European Patent Specification EP 3 444 337 B1, published December 18, 2024. Title: Method of cleaning. Applicant: The Procter & Gamble Company. The sequence listing filed with the application follows.

SEQUENCE LISTING (8 sequences)

SEQ ID NO: 1 - protein, 616 aa, Myceliophthora thermophila
MKSFISAATLLVGILTPSVAAAPPSTPEQRDLLVPITEREEAAVKARQQSCNTPSNRACWTDGYDINTDYEVDSPDTGVVRPYTLTLTEVDNWTGPDGVVKEKVMLVNRPTIFADWGDTIQVTVINNLETNGTSIHWHGLHQKGTNLHDGANGITECPIPPKGGRKVYRFKAQQYGTSWYHSHFSAQYGNGVVGAIQINGPASLPYDTDLGVFPISDYYYSSADELVELTKNSGAPFSDNVLFNGTAKHPETGEGEYANVTLTPGRRHRLRLINTSVENHFQVSLVNHTMTIIAADMVPVNAMTVDSLFLGVGQRYDVVIEASRTPGNYWFNVTFGGGLLCGGSRNPYPAAIFHYAGAPGGPPTDEGKAPVDHNCLDLPNLKPVVARDVPLSGFAKRPDNTLDVTLDTTGTPLFVWKVNGSAINIDWGRPVVDYVLTQNTSFPPGYNIVEVNGADQWSYWLIENDPGAPFTLPHPMHLHGHDFYVLGRSPDESPASNERHVFDPARDAGLLSGANPVRRDVTMLPAFGWVVLAFRADNPGAWLFHCHIAWHVSGGLGVVYLERADDLRGAVSDADADDLDRLCADWRHYWPTNPYPKSDSGLKHRWVEEGEWLVKA

SEQ ID NO: 2 - protein, 513 aa, Bacillus licheniformis
MKLEKFVDRLPIPQVLQPQSKSKEMTYYEVTMKEFQQQLHRDLPPTRLFGYNGVYPGPTFEVQKHEKVAVKWLNKLPDRHFLPVDHTLHDDGHHEHEVKTVVHLHGGCTPADSDGYPEAWYTKDFHAKGPFFEREVYEYPNEQDATALWYHDHAMAITRLNVYAGLVGLYFIRDREERSLNLPKGEYEIPLLIQDKSFHEDGSLFYPRQPDNPSPDLPDPSIVPAFCGDTILVNGKVWPFAELEPRKYRFRILNASNTRIFELYFDHDITCHQIGTDGGLLQHPVKVNELVIAPAERCDIIVDFSRAEGKTVTLKKRIGCGGQDADPDTDADIMQFRISKPLKQKDTSSLPRILRKRPFYRRHKINALRNLSLGAAVDQYGRPVLLLNNTKWHEPVTETPALGSTEIWSIINAGRAIHPIHLHLVQFMILDHRPFDIERYQENGELVFTGPAVPPAPNEKGLKDTVKVPPGSVTRIIATFAPYSGRYVWHCHILEHEDYDMMRPLEVTDVRHQ

SEQ ID NO: 3 - protein, 325 aa, Streptomyces sviceus
MGALDRRGFNRRVLLGGAAVATSLSLAPEARSDAGPAQAAPGGEVRRIKLYAERLADGQMGYGLEKGRATIPGPLIELNEGDTLHIEFENTMDVRASLHVHGLDYEVSSDGTTLNKSDVEPGGTRTYTWRTHAPGRRSDGTWRAGSAGYWHYHDHVVGTEHGTGGIRKGLYGPVIVRRKGDVLPDATHTIVFNDMLINNRPAHSGPNFEATVGDRVEFVMITHGEYYHTFHMHGHRWADNRTGMLTGPDDPSQVVDNKIVGPADSFGFQVIAGEGVGAGAWMYHCHVQSHSDMGMVGLFLVKKTDGTIPGYEPHEHSGQRAEHHH

SEQ ID NO: 4 - protein, 366 aa, Bjerkandera adusta
MAFKQLAAALSIALALPFSQAAITRRVACPDGVNTATNAACCALFAVRDDIQQNLFDGGECGEEVHESLRLTFHDAIGISPSLAATGKFGGGGADGSIMIFDDIEPNFHANNGVDEIINAQKPFVAKHNMTAGDFIQFAGAVGVSNCPGAPQLSFFLGRPAATQPAPDGLVPEPFDSVTDILNRFADAGGFTTQEVVWLLASHSIAAADHVDPTIPGSPFDSTPEIFDTQFFVETLLKGTLFPGTSGNQGEVESPLAGEIRLQSDADFARDSRTACEWQSFVNNQPRMQVLFKAAMQKLSILGHDLTQMIDCSDVIPVPPSTAVRGSHLPAGNTLDDIEQACASTPFPSLTADPGPATSVAPVPPS

SEQ ID NO: 5 - protein, 367 aa, Bjerkandera adusta
MAFKHLAAVLSIAFSLQAVQGAIIKRVACPDGRHTAINAACCNLFTVRDDIQRNMFDGGKCNDIAHQALRLTFHDAVAFSPALEAEGKFGGNGADGSIITFGNIETNFHPNIGLDEIVEIEKPFIARHNMTPGDFLHFAGAIAVTNCPGAPTISFSLGRPVATRPAPDGLVPEPFHTPDQIFARMLDALEFDPLETTWALIAHTVAAADDIDTSIPRSPFDSTPELFDGQFFIETQLKGTLFPGNGPNKGEVRSPLAGEMRLQSDFLIARDNRSACEWQSFGTDHDKLTNRFQFVLETLAMVGQDPTNMIDCSEVIPIPRNLTSAQIPHFPAGKTIRDVEAACPETPFPRLPTDAGRPTAVAPVPRG

SEQ ID NO: 6 - protein, 474 aa, Bjerkandera adusta
AKLGARQSRTTPLLTNFPGQAPLPSLEQHSTQRGANTLPLDNIQGDILVGMKKQKERFVFFHVNDATSFKTALKTYVPDHITSAQTLISDPSEQPLAFVNLAFSNTGLQALGVTDSLGDAQFPNGQFADASNLGDDLSQWVAPFTGTAIHGVFLIGSDQDSFLDQFENDISTAFGASITEVQALSGSARPGDLAGHEHFGFLDGISQPAVTGWETTVFPGQAVVPPGIILTGRDGDPTTRPSWALDGSFMAFRHFQQKVPEFNAYTLANAIPANSAGNLTQQEGAEFLGARMFGRWKSGAPIDLAPTADDPALGADPQRNNNFDFSDTLTDETKCPFAAHIRKTNPRQDLGGPVNTFHAIRSSIPYGPETSDAELASGVTSQDRGLLFVEYQSVIGNGFRFQQINWVNNAGFPFSKPIAPGIDPIIGQSPTRSTGGLDPLDQTKTFSVPLFVIPKGGEYFFMPSISALTSTIAA

SEQ ID NO: 7 - protein, 364 aa, Ganoderma applanatum
MFSKVFLSLVVLASSVAAAVPTVSRRATCTNGKTTANDACCVWFDVLDDIQENLFHGGQCGEDAHESLRLTFHDAIAFSPALTVAGQFGGGGADGSIIAHSDVELTYPVNDGLDEIIEASRPFAIKHNVSFGDFIQFAGAVGVANCNGGPQLSFFAGRSNDSQPSPPNLVPLPSDSADTILSRFSDAGFDALEVVWLLVSHTVGSQNTVDPSIAGAPFDSTPSDFDAQFFVETMLNGTLVPGDGLHDGQVNSPYPGEFRLQSDFALSRDSRTTCEWQKMIADRANMLQKFEVTMLKMSLLGFNQSALTDCSDVIPTATGTVQDPFIPAGLTVDDLQPACSSSAFPTVTTVAGAATSIPAVPLNS

SEQ ID NO: 8 - protein, 430 aa, Thermobifida fusca
MTEPDTERKGSSRRGFLAGLGAAALTGAGIGMAAGEVLRPLLPDSDPAASPEAEQRLRMAAQRADATAAPQPGISGPAPAFVHVIALDLAEEARKNPDTARDSAAAALRSWTELAARLHEESPHDIAEGAASAGLLPASLMVTVGIGGSLLSAIDAEDRRPDALADLPEFSTDDLHPRWCGGDFMLQVGAEDPMVLTAAVEELVAAAADATAVRWSLRGFRRTAAAARDPDATPRNLMGQIDGTANPAQDHPLFDRTITARPADNPAHAWMDGGSYLVVRRIRMLLTEWRKLDVAARERVIGRRLDTGAPLGSRNETDPVVLSARDEEGEPLIPENAHVRLASPENNLGARMFRRGYSYDQGWRDDGVRDAGLLFMAWQGDPATGFIPVQRSLADQGDALNRYIRHEGSALFAVPAAREGRYLGQDLIEG